European Patent Specification EP 3 987 047 B1, published May 7, 2025. Title: BACTERIAL DELIVERY VEHICLES COMPRISING TRACER NUCLEIC ACID SEQUENCES. Applicant: ELIGO BIOSCIENCE. The sequence listing filed with the application follows.

SEQUENCE LISTING (26 sequences)

SEQ ID NO: 1 - DNA, 12335 bp, Artificial Sequence
  Plasmid pAK272B
ctaatctcttgcccccgcccgtaatagcctccaagagattgaagatagtaaagggcaagagctgattcggcgttgaaggatagcggactttcggtcaaccacaattccccactcgacaaaaccagccgtgcgaataactctgaaagtacaagcaacccaagagggctgagcctaaactcagctaattcctaagtgagctaaagactcgaagtgacagctcttaataaatagagcgggaacgtcgaacggtcgtgaaagtaatagtacaacgggtattaacttactgaggatattgcttgaagctgtaccgttttattgggtgaacgaataagatccagcaattcagccaaagaagctaccaatttttagtttaagagtgtcacgtctgacctcgcgggtagattgccgaacgtagagcttacgagccagcggaaacagtagccgcaggataagtaaggggagtaagtgatcgaacgaatcagaagtgacaatatacttaggctggatctcgtcccgtgaatcccaaccctcaccaactacgagataagaggtaagccaaaaatcgacttggtggcgaccaacgactgttccccccctgtaactaatcgttccgtcaaaacctgacttacttcaaggccaattccaagcgcaaacaataccgtcctagttcttcggttaagtttccgaagtaggagtgagcctacctccgtttgcgtcttgttaccactgacccagctatttactttgtattgcctgcaatcgaatttctgaactctcagatagtggggataacgggaaagttcctatatttgcgaactaacttagccgtccacctcgaagctacctactcacacccaccccgcgcggggtaaataaggcactaatcccagctgagagctggcgtagcacttagccacaagttaattaacagttgtctggtagtttggcggtattaggaagatcctagaagcaaggcagagttagttctaacctaaagccacaaataagacaggttgccaaagcccgccggaaattaaatcttgctcagttcggtaacggagtttccctcccgcgtacttaattcccaataagaaacgcgcccaagtcctatcaggcaaaattcagccccttcccgtgttagaacgagggtaaaaatacaagccgattgaacaagggttgggggcttcaaatcgtcgtttaccccactttacaacggagattaagtagttcaccctatagtacgaagcagaactatttcgaggggcgtgcaataatcgaatcttctgcggttgacttaacacgctagggacgtgccctcgattcaatcgaaggtactcctactcagactgcctcacacccagctagtcactgagcgataaaattgacccgccctctagggaagcgagtacgtcccaaagggctccggacagggctatataggagagtttgatctcgccccgacaactgcaaccctcaactcccttagataatattgttagccgaagttgcacgacccgccgtccacggactgctcttagggtgtggctccttaatctgacaacgtgcaacccctatcgaagtcgattgtttctgcgaaaggtgttgtcctaatagtcccgaaatttggcccttgtaggtgtgaaaccacttagcttcgcgccgtagtcctaaaggcccacctattgactttgtttcgggtagcactaggaatcttaacaatttgaatttggacgtggaacgcgtacaccttaatctccgaataattctagggatttggaagtcctctacgttgacacacctacactgctcgaagtaaatatacgaataacgcgggcctcgcggagccgttccgaatcgtcacgtgttcgtttactgttaattggtggcaaataagcaatatcgtagtccgtcaggcccagccctgttatccacggcgttatttgtcaaattgcgtagaactggattgactgcctgacaatacctaattatcggtacgaagtccccgaatctgtcgggctatttcactaatactttccaaacgccccgtatccaagaagaacgaatttatccacgctcccgtctttgggacgaataccgctacaagtggacagaggatcggtacgggcctctaataaatccaacactctacgccctcttcaagagctagaagaacagggtgcagttggaaagggaattatttcgtaaggcgagccaataccgtaattaattcggaagagttaacacgattggaagtaggaatagtttctaaccacggttactaatcctaataacggaacgctgtctgatagattagtgtcagcgctcggtaccaaagaaaaataaaaagacgctgaaaagcgtctttttatttttcggtccagtgtaactcaggcaaaagcacgtaatattcgtactttcttcctccgtaagcgtcacccacattccttaaagagtgcatgtgcatattttgttatcaataaaaaaggccgcgatttgcggccttattgttcgtcttgccggattacgccccgccctgccactcatcgcagtattgttgtaattcattaagcattctgccgacatggaagccatcacaaacggcatgatgaacttggatcgccagtggcattaacaccttgtcgccttgcgtataatattttcccatagtgaaaacgggggcgaagaagttgtccatatttgctacgtttaaatcaaaactggtgaaactcacccacggattggcactgacgaaaaacatattttcgataaaccctttagggaaatatgctaagttttcaccgtaacacgccacatcttgactatatatgtgtagaaactgccggaaatcgtcgtggtattctgaccagagcgatgaaaacgtttcagtttgctcatggaaaacggtgtaacaagggtgaacactatcccatatcaccagctcaccgtctttcattgccatacgaaactccggatgtgcattcatcaggcgggcaagaatgtgaataaaggccggataaaacttgtgcttatttttctttacggtttttaaaaaggccgtaatatccagctgaacggtttggttataggtgcactgagcaactgactggaatgcctcaaaatgttctttacgatgccattgacttatatcaactgtagtatatccagtgatttttttctccattttagcttccttagcttgcgaaatctcgataactcaaaaaatagtagtgatcttatttcattatggtgaaagttgtcttacgtgcaacattttcgcaaaaagttggcgctttatcaacactgtcggaatgacaaatggttccaattattgaacacccttcggggtgtttttttgtttctggtttcccgaggccggcctgcgctagcggagtgtatactggcttactatgttggcactgatgagggtgtaagtgaagtgcttcatgtggcaggagaaaaaaggctgcatcggtgcgtcagcagaatatgtgatacaggatatattccgcttcctcgctcactgactcgctacgctcggtcgttcgactgtggcgagcggaaatggcttacgaacggggcggagatttcctggaagatgccaggaagatacttaacagggaagtgagagggtcgcggcaaagccgtttttccataggctccgcccccctgacaagcatcacgaaatctgacgctcaaatcagtggtggcgaaacctgacaggactataaagataccaggcgtttccccctggcggctccctcgtgcgctctcctgttcctgcctttcggtttgccggtgtcattcctctgttacggccgagtttgtctcattccacgcctgacactcagttccgggtaggcagttcgctccaagctggactgtatgcacgaaccccccgttcagtccgaccgctgcgccttatccggtaactatcgtcttgagtccaacccggaaagacatgcaaaagcaccactggcagcagccactggtaattgatttagaggagttagtcttgaagtcatgcgccggataaggctaaactgaaaggacaagttttggcgactgcgctcctccaagccagttacctcggttcaaagagttggtagctcagagaaccttcgaaaaaccgccctgcaaggcggttttttcgttttcagagcaagagattacgcgcagaccaaaacgatctcaagaagatcatcttattaatcagataaaatatttctagatttcagtgcaatttatctcttcaaatgtagcaccggcgcgccgtgaccaattattgaaggccgctaacgcggcctttttttgtttctggtatcccgaatggagcgacttctccccaaaaagcctcgctttcagcacctgtcgtttcctttcttttcagagggtattttaaataaaaacattaagttatgacgaagaagaacggaaacgccttaaaccggaaaattttcataaatagcgaaaacccgcgaggtcgccgccccgtaacctgtcggatcaccggaaaggacccgtaaagtgataatgattatcatctacatatcacaacgtgcgtaaagggtaagtatgaaggtcgtgtactccatcgctaccaaattccagaaaacagacgctttcgagcgtcttttttcgttttggtcacgacgtacggtggaagattcgttaccaattgacagctagctcagtcctaggtatatacatacatgcttgtttgtttgtaaactactgttttcattaaagaggagaaaggaagccatgtccatctatcaggagtttgttaacaagtattccctgtctaaaaccctgcgttttgaactgatcccgcagggcaaaactttggaaaacattaaagcgcgtggcctgattctggatgacgaaaaacgtgcaaaggattacaagaaagctaaacagatcatcgacaaatatcaccagttctttatcgaagaaattctgtcgtcggtgtgcatcagtgaggatctgttacagaattattctgatgtatactttaaacttaaaaagtccgatgacgataatctgcaaaaagatttcaagtcagccaaagataccatcaagaaacagatctcagaatatattaaagatagcgaaaagttcaaaaacctgtttaaccaaaacctcattgatgctaagaaaggccaagaatctgacctgatcttatggctgaaacagagcaaagataacggcattgaactgttcaaagctaatagcgacatcaccgatattgatgaagcgctcgaaatcatcaagtctttcaaaggctggacgacgtatttcaaaggttttcatgaaaaccgtaagaatgtatattcgagcaacgatattccgacctctattatttatcgtatcgtggacgacaacctgccgaagtttctggaaaacaaagcgaaatatgaatctctgaaagacaaagcaccggaagctattaactatgaacagatcaagaaagatctggcggaagaactgaccttcgacatcgactataaaacctccgaagttaaccagcgtgttttctcactggacgaggttttcgaaatcgctaatttcaacaattacctgaatcaatctggcatcaccaaattcaacaccattattggtggcaaatttgttaacggcgaaaacaccaagcgtaagggcatcaacgaatacattaacctgtatagccaacaaatcaacgacaaaaccctgaaaaagtataaaatgtccgttctgtttaaacagattttatcggacaccgaatctaaatccttcgtaattgataaactggaagatgatagcgacgttgtcaccacgatgcagagcttttatgagcagattgcggcgttcaaaaccgtggaagagaaatctattaaagaaactctgtccctgctctttgacgacctcaaagcgcagaaactagatctgtctaagatttactttaaaaacgacaaatctctgaccgatctcagtcaacaagttttcgatgactatagcgtgatcggcacggcagttttggaatacatcacccaacaaatcgcgccgaaaaatctggacaacccgtccaagaaggaacaggaactgattgcaaagaaaacagaaaaagctaaatacctgagcttagaaactatcaaactggcacttgaggaatttaataaacatcgtgatattgataaacagtgtcgttttgaggaaattctggcgaactttgcggcaatcccgatgatcttcgacgaaattgctcaaaacaaagacaatctggcgcagatctctatcaagtaccagaatcagggtaagaaagatctgcttcaagcatctgcggaggacgatgtgaaagcaattaaagacttattagatcagacgaataacttattacacaagctcaaaatcttccacatcagccagagcgaggacaaggcgaacattctggataaagatgaacacttctatctggtgttcgaagaatgttacttcgaactggcaaacatcgtccctctctacaataaaatccgcaactacatcacgcagaagccttactctgacgagaaattcaaactgaacttcgaaaacagcacgctggcgaacggctgggataagaacaaagagccggacaacaccgcaatcctgttcatcaaagacgacaaatactatctgggcgtaatgaacaagaagaacaacaagatcttcgacgataaagcgatcaaagaaaacaagggtgaaggctataagaaaatcgtgtacaagctcctgccgggtgcgaataaaatgttaccgaaagtgttcttttccgcgaaaagcatcaaattctacaacccgtctgaggatattctgcgcatccgcaatcatagcacgcacactaaaaacggtagcccgcagaaagggtatgaaaaattcgaatttaatatagaggactgccgtaagttcatcgacttctataaacagagcatttccaaacatccggaatggaaagacttcggcttccgtttctctgacactcagcgctataatagcatcgacgagttctaccgcgaagtggagaatcagggctataaactgaccttcgagaacattagtgagtcgtacatcgactccgttgtgaatcagggtaaactgtacctgtttcagatctataataaagactttagcgcgtacagcaaaggccgtccgaatctgcacaccctttactggaaagcattatttgacgaacgtaacctgcaagatgtggtgtataaactgaacggtgaggcggaacttttctaccgtaaacagagtatcccgaagaaaatcacgcatccggcaaaagaagctattgccaacaaaaacaaagacaacccgaagaaagaatcagtattcgaatatgacctgatcaaagataaacgtttcaccgaagataagttctttttccactgtccgattaccatcaacttcaaatctagcggtgcgaacaagttcaacgatgaaattaacttattactgaaagagaaagctaatgacgtacacatcttatctattgatcgcggtgaacgtcatttagcatactatacactggtagatggtaaaggtaatattattaaacaggatactttcaatattatcggtaatgaccgtatgaaaaccaactatcacgataagctggcggcgatcgaaaaagatcgtgattctgcgcgtaaagattggaagaaaattaacaatatcaaagaaatgaaagaaggctatctgagccaagtggtgcacgagatcgcaaaactggtgattgaatataacgctatcgtggttttcgaagatctgaactttggttttaaacgtggtcgcttcaaagtagaaaaacaggtgtaccaaaaactggaaaaaatgctgattgaaaaactgaactatctggtttttaaagacaacgaatttgacaaaacgggtggcgtactccgtgcctatcagctgaccgctccgttcgaaacgttcaagaaaatgggtaaacaaacggggattatctattatgtgccagctggtttcacctccaagatttgtccagttacgggcttcgttaaccagctgtacccgaaatacgagagcgttagcaaatctcaagaatttttcagcaaattcgacaagatctgctataatctggataaaggctatttcgagttcagcttcgattacaaaaacttcggcgataaagcggctaaaggtaagtggactattgctagctttggtagccgtctgattaactttcgcaactccgacaaaaaccataattgggacacgcgtgaagtgtatccgaccaaagaactggaaaaattactgaaagactattccatcgaatatggtcatggggagtgcattaaagcggcgatttgcggtgaatccgataagaaatttttcgccaaactgaccagcgtgcttaacaccattctgcaaatgcgtaattctaaaacgggtacggagctggactacctgatttctccggtagccgacgttaacggcaacttcttcgattctcgtcaagcaccgaaaaatatgccacaagacgcggatgccaacggtgcataccatatcggcttaaaaggcttaatgttattaggccgtatcaagaataatcaggagggcaagaaattaaatctggttatcaaaaacgaagaatacttcgagttcgttcagaatcgtaacaattaatgtatgcttaagcagctcggtaccaaagacgaacaataagacgctgaaaagcgtcttttttcgttttggtcctgttgcggcgcgatagtgtgaacatgctatagacttctggtgctacccgactgacaattaatcatccggctcgtataatgctagcaatttctactgttgtagatcatgacaacggacagcagttatacgtctaagaactttaaataatttctactgttgtagattcgagacgaacaataaggcctccctaacggggggccttttttattgataacaaaagtaacttcgagcttgtctacctcctagcaccattattgcaattaataaacaactaacggacaattctacctaacagttttcatatatgacgagcagttaagtgatgagtaaaggtgaggaattatttactggtgttgttccgatcttagttgaactggacggcgatgttaacggtcataaattcagtgttcgtggtgaaggtgaaggtgatgcaaccaacggtaagctgaccctgaaattcatctgcactactggaaaattaccagtaccgtggcctactctggtgactaccctgacctatggtgttcagtgtttttctcgttaccctgaccacatgaagcaacatgatttcttcaaatctgcaatgccggaaggttatgtacaggagcgcaccatttctttcaaagacgatggcacgtataaaacccgtgcagaggttaaatttgaaggtgacactctggtgaatcgtattgaactgaaaggcattgatttcaaagaggacggcaatattttaggccacaaactggaatataacttcaactcccataacgtttacatcaccgcagacaaacagaagaacggtatcaaagctaacttcaaaattcgccataacgttgaagatggtagcgtacagctggcggatcattaccaacagaacactccgattggagatgctcctgttttactgccggataaccactacctgtccacccagtctaaactgtcgaaggatccgaacgaaaagcgcgaccacatggtgttattagagttcgttaccgctagtggtatcacgcacggtatggatgaactctacaaataagacgaacaataaggggagcgggaaaccgctccccttttttattgataacaaaagtaaattgcacgctgatagtctcccaattgcgaaggaccaaaacgaaaaaacaccctttcgggtgtcttttctggaatttggtaccgagtactaggtatcgtgtaagtagcgaaggcccgtacgcgagataaactgctaggcaaccgcgactctacgactggtgctcgatttaatttcgctgacgtaaagaaattatcggcagtgcgtcaactgccgtatctttatcttaattaggtagttggacaagcccttgaaagaaatagcaagagcctgcctctctattgaagtcacggcgaaagtcgggtagaaatcaaagaaagcagaaattaaatcggagtaacactaaggtgggataactccgtaactgactacgcctttctctagactttacttgaccagatacactgtctttgacacgttgaaggattagagcaatcaaatccaagactggctaagcacgaagcaactcttgagtgttaaaaagttatctcctgtattcgggaagcgggtactagaagattgcagggactccgacgttaagtaaattacaaagtaataagtatcgttcaggatcacgttaccgcaataagaagcgagaataatataatttccgaagtgcttaccccagtagtgactattcctataacccttctgagtgtccggaggcggaaatttgccacgaaagagaaagtatttccccgacaataataaaggggcgctcctcagcttttccacttggttgggtaagctaggcaactctgaaaggagtttcggcgaattgaagccgacagctttgaattgttttaggggcgttattcgagggcaatcggagctaacttcaagactacttctttgttgaatactaaatagtgcaaaggtcgtgtttcctcaaggatactccgctaacaatataggattccaatcagattcagcactggcggtacgggtgttgcggtgaggcgttcgggtttacggctcgaagctagcacggtaggaagcctgacaatcaccaagcaaaagggccgtcgaaggcccacaagatacgaaagctctcgaagccttatccttgaccgatccacctatttaggcagttacgcacaaaagctacccaataatccgtgacaggcacaatatcacggaacaaaaccgaaaactctcgtacacggttaggttttcgctaggaagaataaacctctatcttgattataagaaggctccccaagcacccccaaaaccgaaatagcggtttgcaataagggacaagttacgagtgtagacacgcagaattatccagcctttagtctttaggaaggcaaagctattgtacgcggtagccgtcgtagcaatttaccaactgtagaattattggacacacgtaggaagggcttacagttgaagtttaataaggtcacacgcaaaaccgctaaggaataatcgcaccgttagcgaaagaatatttcagagcggttagtaaaggttgagtaaagtgagattccaaagtgagcctttataaaaagtaaagagctataataaaaccgtcgagcagaaaacaatcgcctgaaatctcaagcacgttgccctttctaacgtcgctaaggtttcgtaaacccgtttgattaggaagaagaataagtaacccgattaggtttgagatcgcgggttatcggtttggattaaaagtggataccagcggagtcaacgccgacgcaaacgtacagtgatccaatcctgttgcacggtcaagcacaatcagctcgcaagatcttggaatagtgtgcccaacagtttagttgagggccacgttccgactacaagttgcttcaagaggggaatttggatttggcaatagccccccgtttctacctcaagaggcgacgagtattaaccgcgccagctgtcggcacaagggccaaagaagattccaatttcttattcccgaataacctccgaatccctgcgggaaaatcaccgaccgaatagcctagaagcaagggggaacagataggtataattagcttaagagagtaccagccgtgacaacagcgtagtaaccacaaacttacgctggggcttctttggcggatttttacagatactaacaaggtgatttgaagtaccttagttgaggatttaaacgcgctatccggtaatctccaaattgggaaataccgttcaaagagggctagaattacttaaaagccttcacaccgcctgcgctatacgcgcccactctcccgtttatccgtccaagcggaagcagggcgatcctccgctaagatattcttacgtgtaacgtagctaagtatcccaaatagctggcgtacgcgttgaacaccgcctagaggatcgtgactcgccggacgagcgtgttattggggacttacgccagcgtagactacaacgcgcccagattaaccctgcacgtattgccttgaataacgtactaatctctccggctctcgacaatctatcgagcgactcgattatcaacgggtgtcttgcagtt

SEQ ID NO: 2 - DNA, 30 bp, Artificial Sequence
  Barcode B1
accaaacgacactcttccggcgaatcgcgc

SEQ ID NO: 3 - DNA, 30 bp, Artificial Sequence
  Barcode B2
agcaccccttcgcccccgtcctcgtgtgtt

SEQ ID NO: 4 - DNA, 30 bp, Artificial Sequence
  Barcode B3
agccggaggtaggacaggtgtccgcacagg

SEQ ID NO: 5 - DNA, 30 bp, Artificial Sequence
  Barcode B4
cgcgatgagatggattcccgaccttccgga

SEQ ID NO: 6 - DNA, 30 bp, Artificial Sequence
  Barcode B5
cgctcgctgctcataatctgcgggtggcac

SEQ ID NO: 7 - DNA, 30 bp, Artificial Sequence
  Barcode B6
cggcacgctgtattgtccaagcgccaagca

SEQ ID NO: 8 - DNA, 30 bp, Artificial Sequence
  Barcode B7
ctgcggacggcggctcgcggttagcccaat

SEQ ID NO: 9 - DNA, 41 bp, Artificial Sequence
  primer that binds to a common region of the pAK272B plasmid backbone
acggaacgctgtctgatagattagtgtcagcgctcggtacc

SEQ ID NO: 10 - DNA, 41 bp, Artificial Sequence
  primer that binds specifically to B1
tgcacatgcactctttaaggaatgtgggtgacgcttacgga

SEQ ID NO: 11 - DNA, 30 bp, Artificial Sequence
  primer that binds specifically to B2
aacacacgaggacgggggcgaaggggtgct

SEQ ID NO: 12 - DNA, 30 bp, Artificial Sequence
  primer that binds specifically to B3
cctgtgcggacacctgtcctacctccggct

SEQ ID NO: 13 - DNA, 30 bp, Artificial Sequence
  primer that binds specifically to B4
tccggaaggtcgggaatccatctcatcgcg

SEQ ID NO: 14 - DNA, 30 bp, Artificial Sequence
  primer that binds specifically to B5
gtgccacccgcagattatgagcagcgagcg

SEQ ID NO: 15 - DNA, 30 bp, Artificial Sequence
  primer that binds specifically to B6
tgcttggcgcttggacaatacagcgtgccg

SEQ ID NO: 16 - DNA, 30 bp, Artificial Sequence
  primer that binds specifically to B7
attgggctaaccgcgagccgccgtccgcag

SEQ ID NO: 17 - protein, 29 aa, Artificial Sequence
  Figure 3 (amino acid representation)
KVKDAEDQLGARVGIELDLNSGKILESFR

SEQ ID NO: 18 - DNA, 30 bp, Artificial Sequence
  Sequence encoding ARVGYIELDL
gcacgagtgggttacatcgaactggatctc

SEQ ID NO: 19 - protein, 10 aa, Artificial Sequence
  Sequence encoded by SEQ ID NO: 18
ARVGYIELDL

SEQ ID NO: 20 - DNA, 27 bp, Artificial Sequence
  Sequence encoding RVGYIELDL
cgtgttggttatattgaacttgatctt

SEQ ID NO: 21 - protein, 9 aa, Artificial Sequence
  Sequence encoded by SEQ ID NO: 20
RVGYIELDL

SEQ ID NO: 22 - DNA, 30 bp, Artificial Sequence
  Barcode B8
gatgacagcggcacacggacacaagcgtca

SEQ ID NO: 23 - DNA, 30 bp, Artificial Sequence
  Barcode B9
gtcccgtggatggctcgaagcctaaccgag

SEQ ID NO: 24 - DNA, 30 bp, Artificial Sequence
  Barcode B10
taacacggagagccatcctcagcccgtcag

SEQ ID NO: 25 - DNA, 30 bp, Artificial Sequence
  Barcode B11
tcctactccaccggcagccttagcgtttgg

SEQ ID NO: 26 - DNA, 30 bp, Artificial Sequence
  Barcode B12
tgcgcgttcttagcgtgtgagcggcctcga